European Patent Application EP 4 151 721 A1, published March 22, 2023. Title: T CELL, PREPARATION METHOD FOR SAME, AND APPLICATIONS THEREOF. Applicant: BENETHERA(BEIJING) BIOTECHNOLOGY CO., LTD. The sequence listing filed with the application follows.

SEQUENCE LISTING (48 sequences)

SEQ ID NO: 1 - DNA, 20 bp, Artificial Sequence
  primer
catcccactgtgacgagatg

SEQ ID NO: 2 - DNA, 19 bp, Artificial Sequence
  primer
acttggagcacaggggtct

SEQ ID NO: 3 - RNA, 58 nt, Artificial Sequence
  shRNA
ccggcaacaagaugaagagcaccaacucgaguuggugcucuucaucuuguuguuuuug

SEQ ID NO: 4 - RNA, 59 nt, Artificial Sequence
  shRNA
aauucaaaaacaacaagaugaagagcaccaacucgaguuggugcucuucaucuuguugg

SEQ ID NO: 5 - RNA, 58 nt, Artificial Sequence
  shRNA
ccggccgcuaaugaagccauauaaacucgaguuuauauggcuucauuagcgguuuuug

SEQ ID NO: 6 - RNA, 58 nt, Artificial Sequence
  shRNA
aauucaaaaaccgcuaaugaagccauauaaacucgaguuuauauggcuucauuagcgg

SEQ ID NO: 7 - RNA, 58 nt, Artificial Sequence
  shRNA
ccgggcaguagguaagaaguuauuacucgaguaauaacuucuuaccuacugcuuuuug

SEQ ID NO: 8 - RNA, 58 nt, Artificial Sequence
  shRNA
aauucaaaaagcaguagguaagaaguuauuacucgaguaauaacuucuuaccuacugc

SEQ ID NO: 9 - RNA, 59 nt, Artificial Sequence
  shRNA
ccggcacaaccaccaacucggucaaacucgaguuugaccgaguugagguuguguuuuug

SEQ ID NO: 10 - RNA, 58 nt, Artificial Sequence
  shRNA
aauucaaaaacacaaccucaacucggucaaacucgaguuugaccgaguugagguugug

SEQ ID NO: 11 - RNA, 60 nt, Artificial Sequence
  shRNA
ccgggcccuugcuuaucuguauaaucucgagauuauacagauaagcaagggcuuuuuugg

SEQ ID NO: 12 - RNA, 59 nt, Artificial Sequence
  shRNA
aauucaaaaaagcccuugcuuaucuguauaaucucgagauuauacagauaagcaagggc

SEQ ID NO: 13 - RNA, 58 nt, Artificial Sequence
  shRNA
ccggcggagugaacaugcagcauuucucgagaaaugcugcauguucacuccguuuuug

SEQ ID NO: 14 - RNA, 58 nt, Artificial Sequence
  shRNA
aauucaaaaacggagugaacaugcagcauuucucgagaaaugcugcauguucacuccg

SEQ ID NO: 15 - RNA, 58 nt, Artificial Sequence
  shRNA
ccgggcacaucuucacggugaacaacucgaguuguucaccgugaagaugugguuuuug

SEQ ID NO: 16 - RNA, 58 nt, Artificial Sequence
  shRNA
aauucaaaaagcacaucuucacggugaacaacucgaguuguucaccgugaagaugugc

SEQ ID NO: 17 - RNA, 58 nt, Artificial Sequence
  shRNA
ccggccaaggaacuuguuucuauuucucgagaaauagaaacaaguuccuugguuuuug

SEQ ID NO: 18 - RNA, 61 nt, Artificial Sequence
  shRNA
aauucaaaaaccaaggaacuuguuucuauuucucgagaaauagaaacaaagagcuccuugg

SEQ ID NO: 19 - RNA, 58 nt, Artificial Sequence
  shRNA
ccgguaggaacgcaauggauauuaacucgaguuaauauccauugcguuccuauuuuug

SEQ ID NO: 20 - RNA, 59 nt, Artificial Sequence
  shRNA
aauucaaaaauaggaacgcaauggauauuaacucgaguuaauauuccauugcguuccua

SEQ ID NO: 21 - DNA, 23 bp, Artificial Sequence
  primer
catcactgccacccagaagactg

SEQ ID NO: 22 - DNA, 23 bp, Artificial Sequence
  primer
atgccagtgagcttcccgttcag

SEQ ID NO: 23 - DNA, 20 bp, Artificial Sequence
  primer
cggacaggattgacagattg

SEQ ID NO: 24 - DNA, 20 bp, Artificial Sequence
  primer
cggacaggattgacagattg

SEQ ID NO: 25 - DNA, 19 bp, Artificial Sequence
  primer
atggctttaaggcacagcg

SEQ ID NO: 26 - DNA, 20 bp, Artificial Sequence
  primer
cagagcccgaatcatccagc

SEQ ID NO: 27 - DNA, 19 bp, Artificial Sequence
  primer
cccatccccaggagtcttg

SEQ ID NO: 28 - DNA, 21 bp, Artificial Sequence
  primer
accatgactaggggcactgta

SEQ ID NO: 29 - DNA, 22 bp, Artificial Sequence
  primer
cgttttgagtttgaaggcgttt

SEQ ID NO: 30 - DNA, 19 bp, Artificial Sequence
  primer
catcttgcgccaattcccg

SEQ ID NO: 31 - DNA, 20 bp, Artificial Sequence
  primer
gatcggccagagttactccg

SEQ ID NO: 32 - DNA, 21 bp, Artificial Sequence
  primer
tgggtagtcatggtctgtgtc

SEQ ID NO: 33 - DNA, 20 bp, Artificial Sequence
  primer
ggctacctggaccttatggg

SEQ ID NO: 34 - DNA, 19 bp, Artificial Sequence
  primer
gcaggcactaaatgtgacc

SEQ ID NO: 35 - DNA, 21 bp, Artificial Sequence
  primer
atccgagtctcctacgacacc

SEQ ID NO: 36 - DNA, 21 bp, Artificial Sequence
  primer
cagtttggactgcatctcgaa

SEQ ID NO: 37 - DNA, 19 bp, Artificial Sequence
  primer
ggactgcacacaggcattg

SEQ ID NO: 38 - DNA, 20 bp, Artificial Sequence
  primer
gtaccttgcggggaatgagc

SEQ ID NO: 39 - DNA, 22 bp, Artificial Sequence
  primer
tgctgaggtgaacaaaggaaag

SEQ ID NO: 40 - DNA, 21 bp, Artificial Sequence
  primer
tcaaaccgatttgggtcctgt

SEQ ID NO: 41 - DNA, 20 bp, Artificial Sequence
  primer
ggcagcaagttatctcccag

SEQ ID NO: 42 - DNA, 21 bp, Artificial Sequence
  primer
ccacaggatgattggcgtctt

SEQ ID NO: 43 - DNA, 18 bp, Artificial Sequence
  primer
aacgcgacgcacatcaag

SEQ ID NO: 44 - DNA, 20 bp, Artificial Sequence
  primer
ctggtacgcgatcagaaagc

SEQ ID NO: 45 - DNA, 19 bp, Artificial Sequence
  primer
gggtgggctcgtgttacag

SEQ ID NO: 46 - DNA, 25 bp, Artificial Sequence
  primer
ggacgggtaagtaacagagtctcta

SEQ ID NO: 47 - DNA, 28 bp, Artificial Sequence
  primer
atcgctcgagatgtgcacacctaggcca

SEQ ID NO: 48 - DNA, 28 bp, Artificial Sequence
  primer
atcggaattctcaagggcagggattgga